European Patent Application EP 4 424 832 A1, published September 4, 2024. Title: GENE THERAPY WITH THE GENES HOKD AND LDRB FOR CANCER TREATMENT. Applicant: Universidad de Granada. Application EP 22886204.1, filed October 25, 2022. The sequence listing filed with the application follows.

SEQUENCE LISTING (4 sequences)

SEQ ID NO: 1 - DNA, 156 bp, Escherichia coli
  source 1..156: mol_type = genomic DNA
atgaagcagcaaaaggcgatgttaatcgccctgatcgtcatctgtttaaccgtcatagtgacggcactggtaacgaggaaagacctctgcgaggtacgaatccgaaccggccagacggaggtcgctgtcttcacagcttacgaacctgaggagtaa

SEQ ID NO: 2 - DNA, 108 bp, Escherichia coli
  source 1..108: mol_type = genomic DNA
atgacgctcgcgcagtttgccatgactttctggcacgacctggcggcaccgatcctggcgggaattattaccgcagcgattgtcggctggtggcgtaaccggaagtaa

SEQ ID NO: 3 - protein, 51 aa, Escherichia coli
MKQQKAMLIALIVICLTVIVTALVTRKDLCEVRIRTGQTEVAVFTAYEPEE

SEQ ID NO: 4 - protein, 35 aa, Escherichia coli
MTLAQFAMTFWHDLAAPILAGIITAAIVGWWRNRK